European Patent Specification EP 3 555 315 B1, published July 9, 2025. Title: Verfahren und System zum Vervielfältigen einer Nukleinsäure. Applicant: GNA Biosolutions GmbH. The sequence listing filed with the application follows.

SEQUENCE LISTING (10 sequences)

SEQ ID NO: 1 - DNA, 25 bp, Artificial seqence
  synthetische funktionelle Nukleinsäure
agatggtatgtggaagttagattgg

SEQ ID NO: 2 - DNA, 26 bp, Artificial sequence
  synthetische funktionelle Nukleinsäure
tcctggaataatgacgctatgatccc

SEQ ID NO: 3 - DNA, 62 bp, Artificial sequence
  synthetische funktionelle Nukleinsäure
gcagaaagaccaaagcatacataaaaaaaaaaaaaaaaaaaaaaaaaaaaaaaaaaaaaaaa

SEQ ID NO: 4 - DNA, 62 bp, Artificial sequence; identical to SEQ ID NO: 3
  synthetische funktionelle Nukleinsäure

SEQ ID NO: 5 - DNA, 40 bp, Artificial sequence
  synthetische funktionelle Nukleinsäure
  misc_feature (1)..(1): 5'-Thiol-Thymin
nttttttttttttttttttttttttttttttttttttttt

SEQ ID NO: 6 - DNA, 40 bp, Artificial sequence
  synthetische funktionelle Nukleinsäure
  misc_feature (40)..(40): 3'-Thiol-Thymin
tttttttttttttttttttttttttttttttttttttttn

SEQ ID NO: 7 - DNA, 40 bp, Artificial sequence
  synthetische funktionelle Nukleinsäure
aaaaaaaaaaaaaaaaaaaaaaaaaaaaaaaaaaaaaaaa

SEQ ID NO: 8 - DNA, 25 bp, Artificial sequence
  synthetische funktionelle Nukleinsäure
agatggtatgtggaagttagattgg

SEQ ID NO: 9 - DNA, 40 bp, Artificial sequence; identical to SEQ ID NO: 7
  synthetische funktionelle Nukleinsäure

SEQ ID NO: 10 - DNA, 22 bp, Artificial sequence
  synthetische funktionelle Nukleinsäure
atgtatgctttggtctttctgc